European Patent Specification EP 3 778 906 B1, published July 2, 2025. Title: ONCOLYTIC HSV VECTOR. Applicant: University of Pittsburgh - Of the Commonwealth System of Higher Education. The sequence listing filed with the application follows.

SEQUENCE LISTING (16 sequences)

SEQ ID NO: 1 - DNA, 115 bp, Artificial Sequence
  primer
ctagtggcattcaccgcgtgccttatagtaccagggcattcaccgcgtgccttaaggatcctggcattcaccgcgtgccttaatgactgcggcattcaccgcgtgccttagagct

SEQ ID NO: 2 - DNA, 154 bp, Artificial Sequence
  primer
ctagtgcggccgcgtctcgggaccgcactcgttatcgaatagtctgactacaacttagtaccagatcgaatagtctgactacaactaggatcctatcgaatagtctgactacaactatgactgcatcgaatagtctgactacaactctcgagct

SEQ ID NO: 3 - DNA, 29 bp, Artificial Sequence
  primer
tcgaggatcctgtcagtgcgcacgcacac

SEQ ID NO: 4 - DNA, 32 bp, Artificial Sequence
  primer
tcgaggatccaaacacccgaggaaatgaaaag

SEQ ID NO: 5 - DNA, 22 bp, Artificial Sequence
  primer
ccccgctggaactactatgaca

SEQ ID NO: 6 - DNA, 107 bp, Artificial Sequence
  primer
ctaaggcacgcggtgaatgccgcagtcattaaggcacgcggtgaatgccaggatccttaaggcacgcggtgaatgccctggtactataaggcacgcggtgaatgcca

SEQ ID NO: 7 - DNA, 146 bp, Artificial Sequence
  primer
cgagagttgtagtcagactattcgatgcagtcatagttgtagtcagactattcgataggatcctagttgtagtcagactattcgatctggtactaagttgtagtcagactattcgataacgagtgcggtcccgagacgcggccgca

SEQ ID NO: 8 - DNA, 27 bp, Artificial Sequence
  primer
tgcagctagccagacccctcccctcgc

SEQ ID NO: 9 - DNA, 32 bp, Artificial Sequence
  primer
tcgagctagcgctcagcgagcagcaagagttc

SEQ ID NO: 10 - DNA, 19 bp, Artificial Sequence
  primer
gcatcaggaaccccaggtt

SEQ ID NO: 11 - DNA, 20 bp, Artificial Sequence
  probe
ttcagcgccgtcagcgagga

SEQ ID NO: 12 - DNA, 70 bp, Artificial Sequence
  primer
tgcccgtcgcgcgtgtttgatgttaataaataacacataaatttggctggccactagtccagtgtggtgg

SEQ ID NO: 13 - DNA, 73 bp, Artificial Sequence
  primer
ctgaaatgcccccccccccttgcgggcggtccattaaagacaacaaacaaatccccagcatgcctgctattgt

SEQ ID NO: 14 - DNA, 22 bp, Artificial Sequence
  primer
ccccgctggaactactatgaca

SEQ ID NO: 15 - DNA, 19 bp, Artificial Sequence
  primer
gcatcaggaaccccaggtt

SEQ ID NO: 16 - DNA, 20 bp, Artificial Sequence
  probe
ttcagcgccgtcagcgagga